European Patent Specification EP 3 573 614 B1, published November 20, 2024. Title: PHARMACEUTICAL COMPOSITIONS FOR COMBINATION THERAPY. Applicant: GENFIT. The sequence listing filed with the application follows.

SEQUENCE LISTING (22 sequences)

SEQ ID NO: 1 - DNA, 20 bp, artificial
  alpha-SMA forward
ctgacagaggcaccactgaa

SEQ ID NO: 2 - DNA, 20 bp, artificial
  alpha-SMA reverse
catctccagagtccagcaca

SEQ ID NO: 3 - DNA, 20 bp, artificial
  Col1a1 forward
aggcgaacaaggtgacagag

SEQ ID NO: 4 - DNA, 19 bp, artificial
  Col1a1 reverse
gccaggagaaccagcagag

SEQ ID NO: 5 - DNA, 20 bp, artificial
  Col1a2 forward
attggaagccgaggtcccag

SEQ ID NO: 6 - DNA, 20 bp, artificial
  Col1a2 reverse
tttgcccccaggtatgccag

SEQ ID NO: 7 - DNA, 20 bp, artificial
  TGFb1 forward
ttgcttcagctccacagaga

SEQ ID NO: 8 - DNA, 20 bp, artificial
  TGFb1 reverse
tggttgtagagggcaaggac

SEQ ID NO: 9 - DNA, 20 bp, artificial
  TIMP1 forward
attcaaggctgtgggaaatg

SEQ ID NO: 10 - DNA, 20 bp, artificial
  TIMP1 reverse
ctcagagtacgccagggaac

SEQ ID NO: 11 - DNA, 20 bp, artificial
  TIMP2 forward
gcatcacccagaagaagagc

SEQ ID NO: 12 - DNA, 20 bp, artificial
  TIMP2 reverse
gggtcctcgatgtcaagaaa

SEQ ID NO: 13 - DNA, 20 bp, artificial
  MMP2 forward
tccctaagctcatcgcagac

SEQ ID NO: 14 - DNA, 20 bp, artificial
  MMP2 reverse
gcttccaaacttcacgctct

SEQ ID NO: 15 - DNA, 20 bp, artificial
  MMP7 forward
taattggcttcgcaaggaga

SEQ ID NO: 16 - DNA, 22 bp, artificial
  MMP7 reverse
aaggcatgacctagagtgttcc

SEQ ID NO: 17 - DNA, 27 bp, artificial
  CCR2 forward
taatatgttacctcagttcatccacgg

SEQ ID NO: 18 - DNA, 26 bp, artificial
  CCR2 reverse
tgctcttcagctttttacagcctatc

SEQ ID NO: 19 - DNA, 20 bp, artificial
  CCR5 forward
attctccacaccctgtttcg

SEQ ID NO: 20 - DNA, 20 bp, artificial
  CCR5 reverse
gaattcctggaaggtggtca

SEQ ID NO: 21 - DNA, 20 bp, artificial
  GAPDH forward
tatgactccactcacggcaa

SEQ ID NO: 22 - DNA, 20 bp, artificial
  GAPDH reverse
tccacgacatactcagcacc